European Patent Application EP 4 421 095 A1, published August 28, 2024. Title: 抗间皮素纳米抗体及其用途. Applicant: 普米斯生物技术（珠海）有限公司. Application CN. The sequence listing filed with the application follows.

SEQUENCE LISTING (19 sequences)

SEQ ID NO: 1 - protein, 7 aa, synthetic construct
  source 1..7: note = YE-17 CDR1
GTIFSRN

SEQ ID NO: 2 - protein, 7 aa, synthetic construct
  source 1..7: note = YE-17 CDR2
ILNDGTT

SEQ ID NO: 3 - protein, 10 aa, synthetic construct
  source 1..10: note = YE-17 CDR3
GYSDYRGTDY

SEQ ID NO: 4 - protein, 116 aa, synthetic construct
  source 1..116: note = YE-17 VHH
QVQLQESGGGLVQPGGSLRLSCATSGTIFSRNGMGWFRQAPGEQRELVARILNDGTTMYADSVKGRFTISRDNAKNTVLLQMNSLKPEDTAVYYCGYSDYRGTDYWGQGTQVTVSS

SEQ ID NO: 5 - protein, 226 aa, synthetic construct
  source 1..226: note = human IgG1-Fc fragment
DKTHTCPPCPAPEAAGGPSVFLFPPKPKDTLMISRTPEVTCVVVDVSHEDPEVKFNWYVDGVEVHNAKTKPREEQYNSTYRVVSVLTVLHQDWLNGKEYKCKVSNKALPAPIEKTISKAKGQPREPQVYTLPPSRDELTKNQVSLTCLVKGFYPSDIAVEWESNGQPENNYKTTPPVLDSDGSFFLYSKLTVDKSRWQQGNVFSCSVMHEALHNHYTQKSLSLSPG

SEQ ID NO: 6 - protein, 116 aa, synthetic construct
  source 1..116: note = HZ-YE-17-01 VHH
QVQLVESGGGVVQPGGSLRLSCATSGTIFSRNGMGWFRQAPGEQRELVARILNDGTTMYADSVKGRFTISRDNSKNTVLLQMNSLKPEDTAVYYCGYSDYRGTDYWGQGTQVTVSS

SEQ ID NO: 7 - protein, 116 aa, synthetic construct
  source 1..116: note = HZ-YE-17-02 VHH
QVQLVESGGGVVQPGGSLRLSCATSGTIFSRNGMGWFRQAPGKQRELVARILNDGTTMYADSVKGRFTISRDNSKNTVYLQMNSLKPEDTAVYYCGYSDYRGTDYWGQGTQVTVSS

SEQ ID NO: 8 - protein, 116 aa, synthetic construct
  source 1..116: note = HZ-YE-17-03 VHH
QVQLVESGGGVVQPGGSLRLSCATSGTIFSRNGMGWFRQAPGKGLELVARILNDGTTMYADSVKGRFTISRDNSKNTVYLQMNSLKPEDTAVYYCGYSDYRGTDYWGQGTQVTVSS

SEQ ID NO: 9 - protein, 116 aa, synthetic construct
  source 1..116: note = HZ-YE-17-04 VHH
QVQLVESGGGVVQPGGSLRLSCATSGTIFSRNGMGWFRQAPGKGLELVARILNDGTTMYADSVKGRFTISRDNSKNTVYLQMNSLRAEDTAVYYCGYSDYRGTDYWGQGTQVTVSS

SEQ ID NO: 10 - protein, 25 aa, synthetic construct
  source 1..25: note = human immunoglobulin FR1
QVQLVESGGGVVQPGGSLRLSCATS

SEQ ID NO: 11 - protein, 17 aa, synthetic construct
  source 1..17: note = human immunoglobulin FR2 (1)
MGWFRQAPGEQRELVAR

SEQ ID NO: 12 - protein, 17 aa, synthetic construct
  source 1..17: note = human immunoglobulin FR2 (2)
MGWFRQAPGKQRELVAR

SEQ ID NO: 13 - protein, 17 aa, synthetic construct
  source 1..17: note = human immunoglobulin FR2 (3)
MGWFRQAPGKGLELVAR

SEQ ID NO: 14 - protein, 38 aa, synthetic construct
  source 1..38: note = human immunoglobulin FR3 (1)
MYADSVKGRFTISRDNSKNTVLLQMNSLKPEDTAVYYC

SEQ ID NO: 15 - protein, 38 aa, synthetic construct
  source 1..38: note = human immunoglobulin FR3 (2)
MYADSVKGRFTISRDNSKNTVYLQMNSLKPEDTAVYYC

SEQ ID NO: 16 - protein, 38 aa, synthetic construct
  source 1..38: note = human immunoglobulin FR3 (3)
MYADSVKGRFTISRDNSKNTVYLQMNSLRAEDTAVYYC

SEQ ID NO: 17 - protein, 11 aa, synthetic construct
  source 1..11: note = human immunoglobulin FR4
WGQGTQVTVSS

SEQ ID NO: 18 - protein, 449 aa, synthetic construct
  source 1..449: note = heavy chain of amatuximab
QVQLQQSGPELEKPGASVKISCKASGYSFTGYTMNWVKQSHGKSLEWIGLITPYNGASSYNQKFRGKATLTVDKSSSTAYMDLLSLTSEDSAVYFCARGGYDGRGFDYWGSGTPVTVSSASTKGPSVFPLAPSSKSTSGGTAALGCLVKDYFPEPVTVSWNSGALTSGVHTFPAVLQSSGLYSLSSVVTVPSSSLGTQTYICNVNHKPSNTKVDKKVEPKSCDKTHTCPPCPAPELLGGPSVFLFPPKPKDTLMISRTPEVTCVVVDVSHEDPEVKFNWYVDGVEVHNAKTKPREEQYNSTYRVVSVLTVLHQDWLNGKEYKCKVSNKALPAPIEKTISKAKGQPREPQVYTLPPSRDELTKNQVSLTCLVKGFYPSDIAVEWESNGQPENNYKTTPPVLDSDGSFFLYSKLTVDKSRWQQGNVFSCSVMHEALHNHYTQKSLSLSPGK

SEQ ID NO: 19 - protein, 213 aa, synthetic construct
  source 1..213: note = light chain of amatuximab
DIELTQSPAIMSASPGEKVTMTCSASSSVSYMHWYQQKSGTSPKRWIYDTSKLASGVPGRFSGSGSGNSYSLTISSVEAEDDATYYCQQWSKHPLTFGSGTKVEIKRTVAAPSVFIFPPSDEQLKSGTASVVCLLNNFYPREAKVQWKVDNALQSGNSQESVTEQDSKDSTYSLSSTLTLSKADYEKHKVYACEVTHQGLSSPVTKSFNRGEC